European Patent Specification EP 3 518 895 B1, published May 22, 2024. Title: PHOSPHORYLATED TRI-BLOCK COPOLYMERS WITH PATHOGEN VIRULENCE-SUPPRESSING PROPERTIES. Applicant: Alverdy, John et al. The sequence listing filed with the application follows.

SEQUENCE LISTING (2 sequences)

SEQ ID NO: 1 - DNA, 24 bp, Pseudomonas aeruginosa
  misc_feature: PCR forward primer PstS F
cacctatcccaaaacccctggtca

SEQ ID NO: 2 - DNA, 24 bp, Pseudomonas aeruginosa
  misc_feature: PCR reverse primer PstS R
caaacgcttgagtttcatgccttg